European Patent Application EP 4 696 334 A2, published February 18, 2026. Title: FIBROBLAST ACTIVATION PROTEIN TARGETED COMPOUNDS AND USE THEREOF. Applicant: PERSPECTIVE THERAPEUTICS, INC. Application EP, filed May 1, 2024. The sequence listing filed with the application follows.

SEQUENCE LISTING (16 sequences)

SEQ ID NO: 1 - protein, 9 aa, synthetic construct
CTPFEQWWC

SEQ ID NO: 2 - protein, 9 aa, synthetic construct
CTPFEAWWC

SEQ ID NO: 3 - protein, 9 aa, synthetic construct
CTPWEQWWC

SEQ ID NO: 4 - protein, 9 aa, synthetic construct
CTPHEQWWC

SEQ ID NO: 5 - protein, 9 aa, synthetic construct
CTPFEIWWC

SEQ ID NO: 6 - protein, 9 aa, synthetic construct
CTPFEHWWC

SEQ ID NO: 7 - protein, 9 aa, synthetic construct
CTPFEDWWC

SEQ ID NO: 8 - protein, 9 aa, synthetic construct
CTPFEEWWC

SEQ ID NO: 9 - protein, 9 aa, synthetic construct
CTPFEQWYC

SEQ ID NO: 10 - protein, 9 aa, synthetic construct
CTPFEQYWC

SEQ ID NO: 11 - protein, 9 aa, synthetic construct
  MOD_RES 1: note = Dpr (2,3-Diaminoproprionic acid)
  MOD_RES 9: note = Dpr (2,3-Diaminoproprionic acid)
XTPFEQWWX

SEQ ID NO: 12 - protein, 10 aa, synthetic construct
  MOD_RES 5: note = 2-Nal (2-napthylalanine)
SCTPXEQWWC

SEQ ID NO: 13 - protein, 9 aa, synthetic construct
  MOD_RES 4: note = 1-Nal (1-napthylalanine)
CTPXEQWWC

SEQ ID NO: 14 - protein, 9 aa, synthetic construct
  MOD_RES 4: note = Bta (3-benzothienyl-alanine)
CTPXEQWWC

SEQ ID NO: 15 - protein, 9 aa, synthetic construct
  MOD_RES 4: note = 3-Pal (3-pyridyl-alanine)
CTPXEQWWC

SEQ ID NO: 16 - protein, 9 aa, synthetic construct
CWWQEWPTC